European Patent Application EP 4 744 724 A2, published May 20, 2026. Title: Peptides and Methods for Treating Diseases. Applicant: Op-T LLC. Application EP. The sequence listing filed with the application follows.

SEQUENCE LISTING (52 sequences)

SEQ ID NO: 1 - protein, 260 aa, Mus musculus
MIETYSQPSPRSVATGLPASMKIFMYLLTVFLITQMIGSVLFAVYLHRRLDKVEEEVNLHEDFVFIKKLKRCNKGEGSLSLLNCEEMRRQFEDLVKDITLNKEEKKENSFEMQRGDEDPQIAAHVVSEANSNAASVLQWAKKGYYTMKSNLVMLENGKQLTVKREGLYYVYTQVTFCSNREPSSQRPFIVGLWLKPSSGSERILLKAANTHSSSQLCEQQSVHLGGVFELQAGASVFVNVTEASQVIHRVGFSSFGLLKL

SEQ ID NO: 2 - protein, 261 aa, Homo sapiens
MIETYNQTSPRSAATGLPISMKIFMYLLTVFLITQMIGSALFAVYLHRRLDKIEDERNLHEDFVFMKTIQRCNTGERSLSLLNCEEIKSQFEGFVKDIMLNKEETKKENSFEMQKGDQNPQIAAHVISEASSKTTSVLQWAEKGYYTMSNNLVTLENGKQLTVKRQGLYYIYAQVTFCSNREASSQAPFIASLCLKSPGRFERILLRAANTHSSAKPCGQQSIHLGGVFELQPGASVFVNVTDPSQVSHGTGFTSFGLLKL

SEQ ID NO: 3 - protein, 260 aa, Canis lupus familiaris
MIETYSQTAPRSVATGPPVSMKIFMYLLTVFLITQMIGSALFAVYLHRRLDKIEDERNLYEDFVFMKTLQKCNKGEGSLSLLNCEEIKSQFEAFLKEIMLNNEMKKEENIAMQKGDQDPRIAAHVISEASSNPASVLRWAPKGYYTISSNLVSLENGKQLAVKRQGLYYVYAQVTFCSNRAASSQAPFVASLCLHSPSGTERVLLRAASSRGSSKPCGQQSIHLGGVFELHPGASVFVNVTDPSQVSHGTGFTSFGLLKL

SEQ ID NO: 4 - protein, 260 aa, Felis catus
MIETYSQTAPRSVAPGPPVSMKIFMYLLTVFLITQMIGSALFAVYLHRRLDKIEDERNLYEDFVFMKTLQKCNKGEGALSLLNCEEIKSRFEAFLKEIMLNKETKKEKNVAMQKGDQDPRVAAHVISEASSSTASVLQWAPKGYYTISSNLVTLENGKQLAVKRQGLYYIYAQVTFCSNREASSQAPFIASLCLHSPSGSERVLLRAANARSSSKPCGQQSIHLGGVFELHPGASVFVNVTDPSQVSHGTGFTSFGLLKL

SEQ ID NO: 5 - protein, 261 aa, Equus caballus
MIETYSQPSPRSVATGPPVSMKIFMYLLTVFLITQMIVSALFAVYLHRRLDKIEDERNLHEDFVFMKTIQRCNKGEGPLSLLNCEEIRSQFEGFVKDIMLNEEVKKKGENFEMQKGDQEPQIAAHVISEASSKTASVLQWAQKGYYTISNNLVTLENGKQLAVKRQGLYYIYAQVTFCSNREASGQAPFIASLCLRSVSGSERILLRAANTHSSSKPCGQQSIHLGGVFELQPGASVFVNVTDPSQVSHGTGFTSFGLLKL

SEQ ID NO: 6 - protein, 4 aa, synthetic construct
  REGION 1..4: note = Synthetic Peptide
  SITE 1: note = MISC_FEATURE - glycation, alkylation, acetylation, acylation
  SITE 4: note = MISC_FEATURE - amidation
KGYY

SEQ ID NO: 7 - protein, 6 aa, synthetic construct
  REGION 1..6: note = Synthetic Peptide
  SITE 1: note = MISC_FEATURE - glycation, alkylation, acetylation, acylation
  SITE 6: note = MISC_FEATURE - amidation
KKGYYT

SEQ ID NO: 8 - protein, 6 aa, synthetic construct
  REGION 1..6: note = Synthetic Peptide
  SITE 1: note = MISC_FEATURE - glycation, alkylation, acetylation, acylation
  SITE 6: note = MISC_FEATURE - amidation
EKGYYT

SEQ ID NO: 9 - protein, 6 aa, synthetic construct
  REGION 1..6: note = Synthetic Peptide
  SITE 1: note = MISC_FEATURE - glycation, alkylation, acetylation, acylation
  SITE 6: note = MISC_FEATURE - amidation
PKGYYT

SEQ ID NO: 10 - protein, 6 aa, synthetic construct
  REGION 1..6: note = Synthetic Peptide
  SITE 1: note = MISC_FEATURE - glycation, alkylation, acetylation, acylation
  SITE 6: note = MISC_FEATURE - amidation
QKGYYT

SEQ ID NO: 11 - protein, 15 aa, synthetic construct
  REGION 1..15: note = Synthetic Peptide
  SITE 1: note = MISC_FEATURE - glycation, alkylation, acetylation, acylation
  SITE 15: note = MISC_FEATURE - amidation
VLQWAKKGYYTMKSN

SEQ ID NO: 12 - protein, 15 aa, synthetic construct
  REGION 1..15: note = Synthetic Peptide
  SITE 1: note = MISC_FEATURE - glycation, alkylation, acetylation, acylation
  SITE 15: note = MISC_FEATURE - amidation
VLQWAEKGYYTMSNN

SEQ ID NO: 13 - protein, 15 aa, synthetic construct
  REGION 1..15: note = Synthetic Peptide
  SITE 1: note = MISC_FEATURE - glycation, alkylation, acetylation, acylation
  SITE 15: note = MISC_FEATURE - amidation
VLRWAPKGYYTISSN

SEQ ID NO: 14 - protein, 15 aa, synthetic construct
  REGION 1..15: note = Synthetic Peptide
  SITE 1: note = MISC_FEATURE - glycation, alkylation, acetylation, acylation
  SITE 15: note = MISC_FEATURE - amidation
VLQWAPKGYYTISSN

SEQ ID NO: 15 - protein, 15 aa, synthetic construct
  REGION 1..15: note = Synthetic Peptide
  SITE 1: note = MISC_FEATURE - glycation, alkylation, acetylation, acylation
  SITE 15: note = MISC_FEATURE - amidation
VLQWAQKGYYTISNN

SEQ ID NO: 16 - protein, 24 aa, synthetic construct
  REGION 1..24: note = Synthetic Peptide
  SITE 1: note = MISC_FEATURE - glycation, alkylation, acetylation, acylation
NAASVLQWAKKGYYTMKSNLVMLE

SEQ ID NO: 17 - protein, 15 aa, synthetic construct
  REGION 1..15: note = Synthetic Peptide
YKNVKQMAYWLTGKS

SEQ ID NO: 18 - protein, 260 aa, Mus musculus; identical to SEQ ID NO: 1

SEQ ID NO: 19 - protein, 261 aa, Homo sapien; identical to SEQ ID NO: 2

SEQ ID NO: 20 - protein, 4 aa, synthetic construct
  REGION 1..4: note = Synthetic Peptide
  SITE 1: note = MISC_FEATURE - glycation, alkylation, acetylation, acylation
  SITE 4: note = MISC_FEATURE - amidation
KGYY

SEQ ID NO: 21 - protein, 6 aa, synthetic construct
  REGION 1..6: note = Synthetic Peptide
  SITE 1: note = MISC_FEATURE - glycation, alkylation, acetylation, acylation
  SITE 6: note = MISC_FEATURE - amidation
KKGYYT

SEQ ID NO: 22 - protein, 8 aa, synthetic construct
  REGION 1..8: note = Synthetic Peptide
  SITE 1: note = MISC_FEATURE - glycation, alkylation, acetylation, acylation
  SITE 8: note = MISC_FEATURE - amidation
AKKGYYTM

SEQ ID NO: 23 - protein, 8 aa, synthetic construct
  REGION 1..8: note = Synthetic Peptide
  SITE 1: note = MISC_FEATURE - glycation, alkylation, acetylation, acylation
  SITE 8: note = MISC_FEATURE - amidation
AEKGYYTM

SEQ ID NO: 24 - protein, 15 aa, synthetic construct
  REGION 1..15: note = Synthetic Peptide
  SITE 1: note = MISC_FEATURE - glycation, alkylation, acetylation, acylation
  SITE 15: note = MISC_FEATURE - amidation
VLQWAKKGYYTMKSN

SEQ ID NO: 25 - protein, 15 aa, synthetic construct
  REGION 1..15: note = Synthetic Peptide
  SITE 1: note = MISC_FEATURE - glycation, alkylation, acetylation, acylation
  SITE 15: note = MISC_FEATURE - amidation
VLQWAEKGYYTMSNN

SEQ ID NO: 26 - protein, 24 aa, synthetic construct
  REGION 1..24: note = Synthetic Peptide
  SITE 1: note = MISC_FEATURE - glycation, alkylation, acetylation, acylation
  SITE 24: note = MISC_FEATURE - amidation
NAASVLQWAKKGYYTMKSNLVMLE

SEQ ID NO: 27 - protein, 17 aa, synthetic construct
  REGION 1..17: note = Synthetic Peptide
ISQAVHAAHAEINEAGR

SEQ ID NO: 28 - protein, 15 aa, synthetic construct
  REGION 1..15: note = Synthetic Peptide
  SITE 1: note = MISC_FEATURE - glycation, alkylation, acetylation, acylation
  SITE 15: note = MISC_FEATURE - amidation
GLQWAKKGYYTMKSN

SEQ ID NO: 29 - protein, 15 aa, synthetic construct
  REGION 1..15: note = Synthetic Peptide
  SITE 1: note = MISC_FEATURE - glycation, alkylation, acetylation, acylation
  SITE 15: note = MISC_FEATURE - amidation
VGQWAKKGYYTMKSN

SEQ ID NO: 30 - protein, 15 aa, synthetic construct
  REGION 1..15: note = Synthetic Peptide
  SITE 1: note = MISC_FEATURE - glycation, alkylation, acetylation, acylation
  SITE 15: note = MISC_FEATURE - amidation
VLGWAKKGYYTMKSN

SEQ ID NO: 31 - protein, 15 aa, synthetic construct
  REGION 1..15: note = Synthetic Peptide
  SITE 1: note = MISC_FEATURE - glycation, alkylation, acetylation, acylation
  SITE 15: note = MISC_FEATURE - amidation
VLQGAKKGYYTMKSN

SEQ ID NO: 32 - protein, 15 aa, synthetic construct
  REGION 1..15: note = Synthetic Peptide
  SITE 1: note = MISC_FEATURE - glycation, alkylation, acetylation, acylation
  SITE 15: note = MISC_FEATURE - amidation
VLQWGKKGYYTMKSN

SEQ ID NO: 33 - protein, 15 aa, synthetic construct
  REGION 1..15: note = Synthetic Peptide
  SITE 1: note = MISC_FEATURE - glycation, alkylation, acetylation, acylation
  SITE 15: note = MISC_FEATURE - amidation
VLQWAGKGYYTMKSN

SEQ ID NO: 34 - protein, 15 aa, synthetic construct
  REGION 1..15: note = Synthetic Peptide
  SITE 1: note = MISC_FEATURE - glycation, alkylation, acetylation, acylation
  SITE 15: note = MISC_FEATURE - amidation
VLQWAKGGYYTMKSN

SEQ ID NO: 35 - protein, 15 aa, synthetic construct
  REGION 1..15: note = Synthetic Peptide
  SITE 1: note = MISC_FEATURE - glycation, alkylation, acetylation, acylation
  SITE 15: note = MISC_FEATURE - amidation
VLQWAKKGGYTMKSN

SEQ ID NO: 36 - protein, 15 aa, synthetic construct
  REGION 1..15: note = Synthetic peptide
  SITE 1: note = MISC_FEATURE - glycation, alkylation, acetylation, acylation
  SITE 15: note = MISC_FEATURE - amidation
VLQWAKKGYGTMKSN

SEQ ID NO: 37 - protein, 15 aa, synthetic construct
  REGION 1..15: note = Synthetic Peptide
  SITE 1: note = MISC_FEATURE - glycation, alkylation, acetylation, acylation
  SITE 15: note = MISC_FEATURE - amidation
VLQWAKKGYYGMKSN

SEQ ID NO: 38 - protein, 15 aa, synthetic construct
  REGION 1..15: note = Synthetic peptide
  SITE 1: note = MISC_FEATURE - glycation, alkylation, acetylation, acylation
  SITE 15: note = MISC_FEATURE - amidation
VLQWAKKGYYTGKSN

SEQ ID NO: 39 - protein, 17 aa, synthetic construct
  REGION 1..17: note = Synthetic peptide
ISQAVHAAHAEINEAGR

SEQ ID NO: 40 - protein, 15 aa, synthetic construct
  REGION 1..15: note = Synthetic peptide
YVQGKANLKSKLMYT

SEQ ID NO: 41 - protein, 10 aa, synthetic construct
  REGION 1..10: note = Synthetic Peptide
  SITE 1: note = MISC_FEATURE - glycation, alkylation, acetylation, acylation
  SITE 10: note = MISC_FEATURE - amidation
WAKKGYYTMK

SEQ ID NO: 42 - protein, 13 aa, synthetic construct
  REGION 1..13: note = Synthetic peptide
  SITE 1: note = MISC_FEATURE - glycation, alkylation, acetylation, acylation
  SITE 13: note = MISC_FEATURE - amidation
VLQWAKKGYYTMK

SEQ ID NO: 43 - protein, 24 aa, synthetic construct
  REGION 1..24: note = Synthetic peptide
  SITE 1: note = MISC_FEATURE - glycation, alkylation, acetylation, acylation
  SITE 24: note = MISC_FEATURE - amidation
AASVLQWAKKGYYTMKSNLVMLEN

SEQ ID NO: 44 - protein, 6 aa, synthetic construct
  REGION 1..6: note = Synthetic peptide
  SITE 1: note = MISC_FEATURE - glycation, alkylation, acetylation, acylation
  SITE 6: note = MISC_FEATURE - amidation
KGYYTM

SEQ ID NO: 45 - protein, 6 aa, synthetic construct
  REGION 1..6: note = Synthetic peptide
  SITE 1: note = MISC_FEATURE - glycation, alkylation, acetylation, acylation
  SITE 6: note = MISC_FEATURE - amidation
AEKGYY

SEQ ID NO: 46 - protein, 6 aa, synthetic construct
  REGION 1..6: note = Synthetic peptide
  SITE 1: note = MISC_FEATURE - glycation, alkylation, acetylation, acylation
  SITE 6: note = MISC_FEATURE - amidation
AKKGYY

SEQ ID NO: 47 - protein, 6 aa, synthetic construct
  REGION 1..6: note = Synthetic peptide
  SITE 1: note = MISC_FEATURE - glycation, alkylation, acetylation, acylation
  SITE 6: note = MISC_FEATURE - amidation
AKGYYT

SEQ ID NO: 48 - protein, 24 aa, synthetic construct
  REGION 1..24: note = Synthetic peptide
  SITE 1: note = MISC_FEATURE - glycation, alkylation, acetylation, acylation
  SITE 24: note = MISC_FEATURE - amidation
AASVLQWAKKGYYTMKSNLVMLEN

SEQ ID NO: 49 - protein, 15 aa, synthetic construct
  REGION 1..15: note = Synthetic peptide
YKNVKQMAYWLTGKS

SEQ ID NO: 50 - protein, 6 aa, synthetic construct
  REGION 1..6: note = Synthetic peptide
  SITE 1: note = MISC_FEATURE - glycation, alkylation, acetylation, acylation
  SITE 6: note = MISC_FEATURE - amidation
APKGYY

SEQ ID NO: 51 - protein, 6 aa, synthetic construct
  REGION 1..6: note = Synthetic peptide
  SITE 1: note = MISC_FEATURE - glycation, alkylation, acetylation, acylation
  SITE 6: note = MISC_FEATURE - amidation
AQKGYY

SEQ ID NO: 52 - protein, 6 aa, synthetic construct
  REGION 1..6: note = Synthetic peptide
  SITE 1: note = MISC_FEATURE - glycation, alkylation, acetylation, acylation
  SITE 6: note = MISC_FEATURE - amidation
KGYYTI